European Patent Application EP 4 368 639 A1, published May 15, 2024. Title: CD8alpha BINDING POLYPEPTIDE AND USE THEREOF. Applicant: SUZHOU SMARTNUCLIDE BIOPHARMACEUTICAL CO., LTD. The sequence listing filed with the application follows.

SEQUENCE LISTING (59 sequences)

SEQ ID NO: 1 - protein, 125 aa, Artificial Sequence
  C37 VHH
QLQLVESGGGLVQAGGSLRLSCAASGLTFEDYAIGWFRQAPGKEREGISCIRIYDGNTYSAESVKGRFTISSDNAKNQVYLQINTLKPEDTAVYYCAAGSYYSCSVYPDYDMDYWGKGTLVTVSS

SEQ ID NO: 2 - protein, 125 aa, Artificial Sequence
  C37-YHDMS VHH
QLQLVESGGGLVQAGGSLRLSCAASGLTFEDYAIGWFRQAPGKEREGISCIRIYDGNTYYADSVKGRFTISSDNAKNHVYLQMNSLKPEDTAVYYCAAGSYYSCSVYPDYDMDYWGKGTLVTVSS

SEQ ID NO: 3 - protein, 125 aa, Artificial Sequence
  C37-S72R VHH
QLQLVESGGGLVQAGGSLRLSCAASGLTFEDYAIGWFRQAPGKEREGISCIRIYDGNTYSAESVKGRFTISRDNAKNQVYLQINTLKPEDTAVYYCAAGSYYSCSVYPDYDMDYWGKGTLVTVSS

SEQ ID NO: 4 - protein, 125 aa, Artificial Sequence
  C37-T85S VHH
QLQLVESGGGLVQAGGSLRLSCAASGLTFEDYAIGWFRQAPGKEREGISCIRIYDGNTYSAESVKGRFTISSDNAKNQVYLQINSLKPEDTAVYYCAAGSYYSCSVYPDYDMDYWGKGTLVTVSS

SEQ ID NO: 5 - protein, 125 aa, Artificial Sequence
  C37-D109A VHH
QLQLVESGGGLVQAGGSLRLSCAASGLTFEDYAIGWFRQAPGKEREGISCIRIYDGNTYSAESVKGRFTISSDNAKNQVYLQINTLKPEDTAVYYCAAGSYYSCSVYPAYDMDYWGKGTLVTVSS

SEQ ID NO: 6 - protein, 125 aa, Artificial Sequence
  C37-RA VHH
QLQLVESGGGLVQAGGSLRLSCAASGLTFEDYAIGWFRQAPGKEREGISCIRIYDGNTYSAESVKGRFTISRDNAKNQVYLQINTLKPEDTAVYYCAAGSYYSCSVYPAYDMDYWGKGTLVTVSS

SEQ ID NO: 7 - protein, 125 aa, Artificial Sequence
  C37-RSA VHH
QLQLVESGGGLVQAGGSLRLSCAASGLTFEDYAIGWFRQAPGKEREGISCIRIYDGNTYSAESVKGRFTISRDNAKNQVYLQINSLKPEDTAVYYCAAGSYYSCSVYPAYDMDYWGKGTLVTVSS

SEQ ID NO: 8 - protein, 125 aa, Artificial Sequence
  C37-F1 VHH
QLQLVESGGGLVQAGGSLRLSCAASGLTFSDYAIGWFRQAPGKEREGISCIRIYDGNTYYADSVKGRFTISRDNAKNHVYLQMNSLKPEDTAVYYCAAGSYYSCSVYPAYDLDYWGKGTLVTVSS

SEQ ID NO: 9 - protein, 125 aa, Artificial Sequence
  C37H VHH
QVQLVESGGGLVQPGGSLRLSCAASGLTFSDYAIGWFRQAPGKEREGISCIRIYDGNTYYADSVKGRFTISRDNSKNHVYLQMNSLRAEDTAVYYCAAGSYYSCSVYPAYDLDYWGKGTLVTVSS

SEQ ID NO: 10 - protein, 125 aa, Artificial Sequence
  C37-H1 VHH
QVQLVESGGGLVQPGGSLRLSCAASGLTFSDYAIGWFRQAPGKEREGISCIRIYDGRTYYADSVKGRFTISRDNSKNHVYLQMNSLRAEDTAVYYCAAGSYYSCSVYPAYDLDYWGQGTLVTVSS

SEQ ID NO: 11 - protein, 125 aa, Artificial Sequence
  C37-H2 VHH
QVQLVESGGGLVQPGGSLRLSCAASGLTFSDYAIGWFRQAPGKEREGISCIRIYDRNTYYADSVKGRFTISRDNSKNHVYLQMNSLRAEDTAVYYCAAGSYYSCSVYPAYDLDYWGQGTLVTVSS

SEQ ID NO: 12 - protein, 125 aa, Artificial Sequence
  C37-H3 VHH
QVQLVESGGGLVQPGGSLRLSCAASGLTFSDYAIGWFRQAPGKEREGISCIRIYDGNTYYADSVKGRFTISRDNAKNHVYLQMNSLRAEDTAVYYCAAGSYYSCSVYPAYDLDYWGKGTLVTVSS

SEQ ID NO: 13 - protein, 125 aa, Artificial Sequence
  C37-H4 VHH
QVQLVESGGGLVQPGGSLRLSCAASGLTFSDYAIGWFRQAPGKEREGISCIRIYDGNTYYADSVKGRFTISRDNSKNHVYLQMNSLKPEDTAVYYCAAGSYYSCSVYPAYDLDYWGKGTLVTVSS

SEQ ID NO: 14 - protein, 125 aa, Artificial Sequence
  C37-YHDMS VHH; C37-S72R VHH; C37-T85S VHH; C37-D109A VHH; C37-RA VHH; C37-RSA VHH; C37-F1 VHH; C37H VHH; C37-H1 VHH; C37-H2 VHH; C37-H3 VHH; C37-H4 VHH
  misc_feature (2)..(2): Xaa = Leu or Val
  misc_feature (14)..(14): Xaa = Ala or Pro
  misc_feature (30)..(30): Xaa = Glu or Ser
  misc_feature (56)..(56): Xaa = Gly or Arg
  misc_feature (57)..(57): Xaa = Asn or Arg
  misc_feature (60)..(60): Xaa = Ser or Tyr
  misc_feature (62)..(62): Xaa = Asp or Glu
  misc_feature (72)..(72): Xaa = Arg or Ser
  misc_feature (75)..(75): Xaa = Ala or Ser
  misc_feature (78)..(78): Xaa = His or Gln
  misc_feature (83)..(83): Xaa = Ile or Met
  misc_feature (85)..(85): Xaa = Ser or Thr
  misc_feature (87)..(87): Xaa = Lys or Arg
  misc_feature (88)..(88): Xaa = Ala or Pro
  misc_feature (109)..(109): Xaa = Ala or Asp
  misc_feature (112)..(112): Xaa = Leu or Met
  misc_feature (117)..(117): Xaa = Lys or Gln
QXQLVESGGGLVQXGGSLRLSCAASGLTFXDYAIGWFRQAPGKEREGISCIRIYDXXTYXAXSVKGRFTISXDNXKNXVYLQXNXLXXEDTAVYYCAAGSYYSCSVYPXYDXDYWGXGTLVTVSS

SEQ ID NO: 15 - protein, 125 aa, Artificial Sequence
  C37-S72R VHH; C37-T85S VHH; C37-D109A VHH; C37-RA VHH; C37-RSA VHH
  misc_feature (72)..(72): Xaa = Arg or Ser
  misc_feature (85)..(85): Xaa = Ser or Thr
  misc_feature (109)..(109): Xaa = Ala or Asp
QLQLVESGGGLVQAGGSLRLSCAASGLTFEDYAIGWFRQAPGKEREGISCIRIYDGNTYSAESVKGRFTISXDNAKNQVYLQINXLKPEDTAVYYCAAGSYYSCSVYPXYDMDYWGKGTLVTVSS

SEQ ID NO: 16 - protein, 125 aa, Artificial Sequence
  C37-F1 VHH; C37H VHH; C37-H1 VHH; C37-H2 VHH; C37-H3 VHH; C37-H4 VHH
  misc_feature (2)..(2): Xaa = Leu or Val
  misc_feature (14)..(14): Xaa = Ala or Pro
  misc_feature (56)..(56): Xaa = Gly or Arg
  misc_feature (57)..(57): Xaa = Asn or Arg
  misc_feature (75)..(75): Xaa = Ala or Ser
  misc_feature (87)..(87): Xaa = Lys or Arg
  misc_feature (88)..(88): Xaa = Ala or Pro
  misc_feature (117)..(117): Xaa = Lys or Gln
QXQLVESGGGLVQXGGSLRLSCAASGLTFSDYAIGWFRQAPGKEREGISCIRIYDXXTYYADSVKGRFTISRDNXKNHVYLQMNSLXXEDTAVYYCAAGSYYSCSVYPAYDLDYWGXGTLVTVSS

SEQ ID NO: 17 - protein, 7 aa, Artificial Sequence
  C37-YHDMS CDR1; C37-S72R CDR1; C37-T85S CDR1; C37-D109A CDR1; C37-RA CDR1; C37-RSA CDR1
GLTFEDY

SEQ ID NO: 18 - protein, 7 aa, Artificial Sequence
  C37-F1 CDR1; C37H CDR1; C37-H1 CDR1; C37-H2 CDR1; C37-H3 CDR1; C37-H4 CDR1
GLTFSDY

SEQ ID NO: 19 - protein, 7 aa, Artificial Sequence
  C37-YHDMS CDR1; C37-S72R CDR1; C37-T85S CDR1; C37-D109A CDR1; C37-RA CDR1; C37-RSA CDR1; C37-F1 CDR1; C37H CDR1; C37-H1 CDR1; C37-H2 CDR1; C37-H3 CDR1; C37-H4 CDR1
  misc_feature (5)..(5): Xaa = Glu or Ser
GLTFXDY

SEQ ID NO: 20 - protein, 6 aa, Artificial Sequence
  C37-YHDMS CDR2; C37-S72R CDR2; C37-T85S CDR2; C37-D109A CDR2; C37-RA CDR2; C37-RSA CDR2; C37-F1 CDR2; C37H CDR2; C37-H3 CDR2; C37-H4 CDR2
RIYDGN

SEQ ID NO: 21 - protein, 6 aa, Artificial Sequence
  C37-H1 CDR2
RIYDGR

SEQ ID NO: 22 - protein, 6 aa, Artificial Sequence
  C37-H2 CDR2
RIYDRN

SEQ ID NO: 23 - protein, 6 aa, Artificial Sequence
  C37-YHDMS CDR2; C37-S72R CDR2; C37-T85S CDR2; C37-D109A CDR2; C37-RA CDR2; C37-RSA CDR2; C37-F1 CDR2; C37H CDR2; C37-H3 CDR2; C37-H4 CDR2; C37-H1 CDR2; C37-H2 CDR2
  misc_feature (5)..(5): Xaa = Gly or Arg
  misc_feature (6)..(6): Xaa = Asn or Arg
RIYDXX

SEQ ID NO: 24 - protein, 16 aa, Artificial Sequence
  C37-YHDMS CDR3; C37-S72R CDR3; C37-T85S CDR3
GSYYSCSVYPDYDMDY

SEQ ID NO: 25 - protein, 16 aa, Artificial Sequence
  C37-D109A CDR3; C37-RA CDR3; C37-RSA CDR3
GSYYSCSVYPAYDMDY

SEQ ID NO: 26 - protein, 16 aa, Artificial Sequence
  C37-F1 CDR3; C37H CDR3; C37-H1 CDR3; C37-H2 CDR3; C37-H3 CDR3; C37-H4 CDR3
GSYYSCSVYPAYDLDY

SEQ ID NO: 27 - protein, 16 aa, Artificial Sequence
  C37-YHDMS CDR3; C37-S72R CDR3; C37-T85S CDR3; C37-D109A CDR3; C37-RA CDR3; C37-RSA CDR3; C37-F1 CDR3; C37H CDR3; C37-H1 CDR3; C37-H2 CDR3; C37-H3 CDR3; C37-H4 CDR3
  misc_feature (11)..(11): Xaa = Ala or Asp
  misc_feature (14)..(14): Xaa = Leu or Met
GSYYSCSVYPXYDXDY

SEQ ID NO: 28 - protein, 16 aa, Artificial Sequence
  C37-YHDMS CDR3; C37-S72R CDR3; C37-T85S CDR3; C37-D109A CDR3; C37-RA CDR3; C37-RSA CDR3
  misc_feature (11)..(11): Xaa = Ala or Asp
GSYYSCSVYPXYDMDY

SEQ ID NO: 29 - protein, 126 aa, Artificial Sequence
  C37H-C VHH
QVQLVESGGGLVQPGGSLRLSCAASGLTFSDYAIGWFRQAPGKEREGISCIRIYDGNTYYADSVKGRFTISRDNSKNHVYLQMNSLRAEDTAVYYCAAGSYYSCSVYPAYDLDYWGKGTLVTVSSC

SEQ ID NO: 30 - protein, 128 aa, Artificial Sequence
  C37H-VDC VHH
QVQLVESGGGLVQPGGSLRLSCAASGLTFSDYAIGWFRQAPGKEREGISCIRIYDGNTYYADSVKGRFTISRDNSKNHVYLQMNSLRAEDTAVYYCAAGSYYSCSVYPAYDLDYWGKGTLVTVSSVDC

SEQ ID NO: 31 - protein, 128 aa, Artificial Sequence
  C37H-GSC VHH
QVQLVESGGGLVQPGGSLRLSCAASGLTFSDYAIGWFRQAPGKEREGISCIRIYDGNTYYADSVKGRFTISRDNSKNHVYLQMNSLRAEDTAVYYCAAGSYYSCSVYPAYDLDYWGKGTLVTVSSGSC

SEQ ID NO: 32 - protein, 128 aa, Artificial Sequence
  C37H-GGC VHH
QVQLVESGGGLVQPGGSLRLSCAASGLTFSDYAIGWFRQAPGKEREGISCIRIYDGNTYYADSVKGRFTISRDNSKNHVYLQMNSLRAEDTAVYYCAAGSYYSCSVYPAYDLDYWGKGTLVTVSSGGC

SEQ ID NO: 33 - protein, 141 aa, Artificial Sequence
  C37-cHis VHH
QLQLVESGGGLVQAGGSLRLSCAASGLTFEDYAIGWFRQAPGKEREGISCIRIYDGNTYSAESVKGRFTISSDNAKNQVYLQINTLKPEDTAVYYCAAGSYYSCSVYPDYDMDYWGKGTLVTVSSGSMDPGGSHHHHHHHH

SEQ ID NO: 34 - protein, 125 aa, Artificial Sequence
  C37-S60Y VHH
QLQLVESGGGLVQAGGSLRLSCAASGLTFEDYAIGWFRQAPGKEREGISCIRIYDGNTYYAESVKGRFTISSDNAKNQVYLQINTLKPEDTAVYYCAAGSYYSCSVYPDYDMDYWGKGTLVTVSS

SEQ ID NO: 35 - protein, 125 aa, Artificial Sequence
  C37-ST-YS VHH
QLQLVESGGGLVQAGGSLRLSCAASGLTFEDYAIGWFRQAPGKEREGISCIRIYDGNTYYAESVKGRFTISSDNAKNQVYLQINSLKPEDTAVYYCAAGSYYSCSVYPDYDMDYWGKGTLVTVSS

SEQ ID NO: 36 - protein, 125 aa, Artificial Sequence
  C37-YDS VHH
QLQLVESGGGLVQAGGSLRLSCAASGLTFEDYAIGWFRQAPGKEREGISCIRIYDGNTYYADSVKGRFTISSDNAKNQVYLQINSLKPEDTAVYYCAAGSYYSCSVYPDYDMDYWGKGTLVTVSS

SEQ ID NO: 37 - protein, 125 aa, Artificial Sequence
  C37-YMS VHH
QLQLVESGGGLVQAGGSLRLSCAASGLTFEDYAIGWFRQAPGKEREGISCIRIYDGNTYYAESVKGRFTISSDNAKNQVYLQMNSLKPEDTAVYYCAAGSYYSCSVYPDYDMDYWGKGTLVTVSS

SEQ ID NO: 38 - protein, 125 aa, Artificial Sequence
  C37-YDMS VHH
QLQLVESGGGLVQAGGSLRLSCAASGLTFEDYAIGWFRQAPGKEREGISCIRIYDGNTYYADSVKGRFTISSDNAKNQVYLQMNSLKPEDTAVYYCAAGSYYSCSVYPDYDMDYWGKGTLVTVSS

SEQ ID NO: 39 - protein, 125 aa, Artificial Sequence
  C37-KL-QQ VHH
QLQLVESGGGLVQAGGSLRLSCAASGLTFEDYAIGWFRQAPGKEREGISCIRIYDGNTYSAESVKGRFTISSDNAKNQVYLQINTLKPEDTAVYYCAAGSYYSCSVYPDYDMDYWGQGTQVTVSS

SEQ ID NO: 40 - protein, 125 aa, Artificial Sequence
  C37-D111A VHH
QLQLVESGGGLVQAGGSLRLSCAASGLTFEDYAIGWFRQAPGKEREGISCIRIYDGNTYSAESVKGRFTISSDNAKNQVYLQINTLKPEDTAVYYCAAGSYYSCSVYPDYAMDYWGKGTLVTVSS

SEQ ID NO: 41 - protein, 125 aa, Artificial Sequence
  C37-D31Y VHH
QLQLVESGGGLVQAGGSLRLSCAASGLTFEYYAIGWFRQAPGKEREGISCIRIYDGNTYSAESVKGRFTISSDNAKNQVYLQINTLKPEDTAVYYCAAGSYYSCSVYPDYDMDYWGKGTLVTVSS

SEQ ID NO: 42 - protein, 125 aa, Artificial Sequence
  C37-M112L VHH
QLQLVESGGGLVQAGGSLRLSCAASGLTFEDYAIGWFRQAPGKEREGISCIRIYDGNTYSAESVKGRFTISSDNAKNQVYLQINTLKPEDTAVYYCAAGSYYSCSVYPDYDLDYWGKGTLVTVSS

SEQ ID NO: 43 - protein, 125 aa, Artificial Sequence
  C37-TMS VHH
QLQLVESGGGLVQAGGSLRLSCAASGLTFEDYAIGWFRQAPGKEREGISCIRIYDGNTYSAESVKGRFTISSDNAKNTVYLQMNSLKPEDTAVYYCAAGSYYSCSVYPDYDMDYWGKGTLVTVSS

SEQ ID NO: 44 - protein, 125 aa, Artificial Sequence
  C37-E30S VHH
QLQLVESGGGLVQAGGSLRLSCAASGLTFSDYAIGWFRQAPGKEREGISCIRIYDGNTYSAESVKGRFTISSDNAKNQVYLQINTLKPEDTAVYYCAAGSYYSCSVYPDYDMDYWGKGTLVTVSS

SEQ ID NO: 45 - protein, 125 aa, Artificial Sequence
  C37-SA VHH
QLQLVESGGGLVQAGGSLRLSCAASGLTFEDYAIGWFRQAPGKEREGISCIRIYDGNTYSAESVKGRFTISSDNAKNQVYLQINSLKPEDTAVYYCAAGSYYSCSVYPAYDMDYWGKGTLVTVSS

SEQ ID NO: 46 - protein, 125 aa, Artificial Sequence
  C37-SR VHH
QLQLVESGGGLVQAGGSLRLSCAASGLTFSDYAIGWFRQAPGKEREGISCIRIYDGNTYSAESVKGRFTISRDNAKNQVYLQINTLKPEDTAVYYCAAGSYYSCSVYPDYDMDYWGKGTLVTVSS

SEQ ID NO: 47 - protein, 125 aa, Artificial Sequence
  C37-SRA VHH
QLQLVESGGGLVQAGGSLRLSCAASGLTFSDYAIGWFRQAPGKEREGISCIRIYDGNTYSAESVKGRFTISRDNAKNQVYLQINTLKPEDTAVYYCAAGSYYSCSVYPAYDMDYWGKGTLVTVSS

SEQ ID NO: 48 - protein, 125 aa, Artificial Sequence
  C37-SRS VHH
QLQLVESGGGLVQAGGSLRLSCAASGLTFSDYAIGWFRQAPGKEREGISCIRIYDGNTYSAESVKGRFTISRDNAKNQVYLQINSLKPEDTAVYYCAAGSYYSCSVYPDYDMDYWGKGTLVTVSS

SEQ ID NO: 49 - protein, 125 aa, Artificial Sequence
  C37-R VHH
QLQLVESGGGLVQAGGSLRLSCAASGLTFEDYAIGWFRQAPGKEREGISCIRIYDGNTYYADSVKGRFTISRDNAKNQVYLQMNSLKPEDTAVYYCAAGSYYSCSVYPDYDMDYWGKGTLVTVSS

SEQ ID NO: 50 - protein, 125 aa, Artificial Sequence
  C37-TRA VHH
QLQLVESGGGLVQAGGSLRLSCAASGLTFEDYAIGWFRQAPGKEREGISCIRIYDGNTYYADSVKGRFTISRDNAKNTVYLQMNSLKPEDTAVYYCAAGSYYSCSVYPAYDMDYWGKGTLVTVSS

SEQ ID NO: 51 - protein, 125 aa, Artificial Sequence
  C37-YDMS-A VHH
QLQLVESGGGLVQAGGSLRLSCAASGLTFEDYAIGWFRQAPGKEREGISCIRIYDGNTYYADSVKGRFTISSDNAKNQVYLQMNSLKPEDTAVYYCAAGSYYSCSVYPAYDMDYWGKGTLVTVSS

SEQ ID NO: 52 - protein, 125 aa, Artificial Sequence
  C37-YDTMS-A VHH
QLQLVESGGGLVQAGGSLRLSCAASGLTFEDYAIGWFRQAPGKEREGISCIRIYDGNTYYADSVKGRFTISSDNAKNTVYLQMNSLKPEDTAVYYCAAGSYYSCSVYPAYDMDYWGKGTLVTVSS

SEQ ID NO: 53 - protein, 125 aa, Artificial Sequence
  C37-YDTMS-R VHH
QLQLVESGGGLVQAGGSLRLSCAASGLTFEDYAIGWFRQAPGKEREGISCIRIYDGNTYYADSVKGRFTISRDNAKNTVYLQMNSLKPEDTAVYYCAAGSYYSCSVYPDYDMDYWGKGTLVTVSS

SEQ ID NO: 54 - protein, 125 aa, Artificial Sequence
  C37-YDMS-SR VHH
QLQLVESGGGLVQAGGSLRLSCAASGLTFSDYAIGWFRQAPGKEREGISCIRIYDGNTYYADSVKGRFTISRDNAKNQVYLQMNSLKPEDTAVYYCAAGSYYSCSVYPDYDMDYWGKGTLVTVSS

SEQ ID NO: 55 - protein, 125 aa, Artificial Sequence
  C37-YDMS-SRA VHH
QLQLVESGGGLVQAGGSLRLSCAASGLTFSDYAIGWFRQAPGKEREGISCIRIYDGNTYYADSVKGRFTISRDNAKNQVYLQMNSLKPEDTAVYYCAAGSYYSCSVYPAYDMDYWGKGTLVTVSS

SEQ ID NO: 56 - protein, 125 aa, Artificial Sequence
  C37-F VHH
QLQLVESGGGLVQAGGSLRLSCAASGLTFSDYAIGWFRQAPGKEREGISCIRIYDGNTYYADSVKGRFTISRDNAKNTVYLQMNSLKPEDTAVYYCAAGSYYSCSVYPAYDLDYWGKGTLVTVSS

SEQ ID NO: 57 - protein, 125 aa, Artificial Sequence
  C37-F2 VHH
QLQLVESGGGLVQAGGSLRLSCAASGLTFSDYAIGWFRQAPGKEREGISCIRIYDGNTYYADSVKGRFTISRDNAKNQVYLQMNSLKPEDTAVYYCAAGSYYSCSVYPAYDLDYWGKGTLVTVSS

SEQ ID NO: 58 - protein, 125 aa, Artificial Sequence
  C37-F4 VHH
QVQLVESGGGLVQAGGSLRLSCAASGLTFSDYAIGWFRQAPGKEREGISCIRIYDGNTYYADSVKGRFTISRDNAKNTVYLQMNSLKPEDTAVYYCAAGSYYSCSVYPAYDLDYWGKGTLVTVSS

SEQ ID NO: 59 - protein, 125 aa, Artificial Sequence
  C37-F5 VHH
QVQLVESGGGLVQPGGSLRLSCAASGLTFSDYAIGWFRQAPGKEREGISCIRIYDGNTYYADSVKGRFTISRDNAKNTVYLQMNSLKPEDTAVYYCAAGSYYSCSVYPAYDLDYWGKGTLVTVSS